European Patent Specification EP 3 334 442 B1, published December 18, 2024. Title: CELLS FOR IMMUNOTHERAPY ENGINEERED FOR TARGETING CD38 ANTIGEN AND FOR CD38 GENE INACTIVATION. Applicant: CELLECTIS. The sequence listing filed with the application follows.

SEQUENCE LISTING (151 sequences)

SEQ ID NO: 1 - DNA, 47 bp, homo sapiens
  CD38ex1-T2 TALEN target
tgaggtgggttggcgactaaggcgcaccggtgggcactgcggggaca

SEQ ID NO: 2 - protein, 936 aa, artificial sequence
  CD38ex1-T2 Left TALEN
MGDPKKKRKVIDYPYDVPDYAIDIADLRTLGYSQQQQEKIKPKVRSTVAQHHEALVGHGFTHAHIVALSQHPAALGTVAVKYQDMIAALPEATHEAIVGVGKQWSGARALEALLTVAGELRGPPLQLDTGQLLKIAKRGGVTAVEAVHAWRNALTGAPLNLTPQQVVAIASNNGGKQALETVQRLLPVLCQAHGLTPEQVVAIASNIGGKQALETVQALLPVLCQAHGLTPQQVVAIASNNGGKQALETVQRLLPVLCQAHGLTPQQVVAIASNNGGKQALETVQRLLPVLCQAHGLTPQQVVAIASNGGGKQALETVQRLLPVLCQAHGLTPQQVVAIASNNGGKQALETVQRLLPVLCQAHGLTPQQVVAIASNNGGKQALETVQRLLPVLCQAHGLTPQQVVAIASNNGGKQALETVQRLLPVLCQAHGLTPQQVVAIASNGGGKQALETVQRLLPVLCQAHGLTPQQVVAIASNGGGKQALETVQRLLPVLCQAHGLTPQQVVAIASNNGGKQALETVQRLLPVLCQAHGLTPQQVVAIASNNGGKQALETVQRLLPVLCQAHGLTPEQVVAIASHDGGKQALETVQRLLPVLCQAHGLTPQQVVAIASNNGGKQALETVQRLLPVLCQAHGLTPEQVVAIASNIGGKQALETVQALLPVLCQAHGLTPQQVVAIASNGGGRPALESIVAQLSRPDPALAALTNDHLVALACLGGRPALDAVKKGLGDPISRSQLVKSELEEKKSELRHKLKYVPHEYIELIEIARNSTQDRILEMKVMEFFMKVYGYRGKHLGGSRKPDGAIYTVGSPIDYGVIVDTKAYSGGYNLPIGQADEMQRYVEENQTRNKHINPNEWWKVYPSSVTEFKFLFVSGHFKGNYKAQLTRLNHITNCNGAVLSVEELLIGGEMIKAGTLTLEEVRRKFNNGEINFAAD

SEQ ID NO: 3 - protein, 942 aa, artificial sequence
  CD38ex1-T2 Right TALEN
MGDPKKKRKVIDKETAAAKFERQHMDSIDIADLRTLGYSQQQQEKIKPKVRSTVAQHHEALVGHGFTHAHIVALSQHPAALGTVAVKYQDMIAALPEATHEAIVGVGKQWSGARALEALLTVAGELRGPPLQLDTGQLLKIAKRGGVTAVEAVHAWRNALTGAPLNLTPQQVVAIASNNGGKQALETVQRLLPVLCQAHGLTPQQVVAIASNGGGKQALETVQRLLPVLCQAHGLTPEQVVAIASHDGGKQALETVQRLLPVLCQAHGLTPEQVVAIASHDGGKQALETVQRLLPVLCQAHGLTPEQVVAIASHDGGKQALETVQRLLPVLCQAHGLTPEQVVAIASHDGGKQALETVQRLLPVLCQAHGLTPQQVVAIASNNGGKQALETVQRLLPVLCQAHGLTPEQVVAIASHDGGKQALETVQRLLPVLCQAHGLTPEQVVAIASNIGGKQALETVQALLPVLCQAHGLTPQQVVAIASNNGGKQALETVQRLLPVLCQAHGLTPQQVVAIASNGGGKQALETVQRLLPVLCQAHGLTPQQVVAIASNNGGKQALETVQRLLPVLCQAHGLTPEQVVAIASHDGGKQALETVQRLLPVLCQAHGLTPEQVVAIASHDGGKQALETVQRLLPVLCQAHGLTPEQVVAIASHDGGKQALETVQRLLPVLCQAHGLTPQQVVAIASNGGGRPALESIVAQLSRPDPALAALTNDHLVALACLGGRPALDAVKKGLGDPISRSQLVKSELEEKKSELRHKLKYVPHEYIELIEIARNSTQDRILEMKVMEFFMKVYGYRGKHLGGSRKPDGAIYTVGSPIDYGVIVDTKAYSGGYNLPIGQADEMQRYVEENQTRNKHINPNEWWKVYPSSVTEFKFLFVSGHFKGNYKAQLTRLNHITNCNGAVLSVEELLIGGEMIKAGTLTLEEVRRKFNNGEINFAAD

SEQ ID NO: 4 - DNA, 49 bp, homo sapiens
  CD38-1 TALEN target
tgcgagttcagcccggtgtccggggacaaaccctgctgccggctctcta

SEQ ID NO: 5 - protein, 970 aa, artificial sequence
  CD38-1 Left TALEN
MGDPKKKRKVIDYPYDVPDYAIDIADLRTLGYSQQQQEKIKPKVRSTVAQHHEALVGHGFTHAHIVALSQHPAALGTVAVKYQDMIAALPEATHEAIVGVGKQWSGARALEALLTVAGELRGPPLQLDTGQLLKIAKRGGVTAVEAVHAWRNALTGAPLNLTPQQVVAIASNGGGKQALETVQRLLPVLCQAHGLTPEQVVAIASNNGGKQALETVQALLPVLCQAHGLTPQQVVAIASHDGGKQALETVQRLLPVLCQAHGLTPQQVVAIASNNGGKQALETVQRLLPVLCQAHGLTPQQVVAIASNIGGKQALETVQRLLPVLCQAHGLTPQQVVAIASNNGGKQALETVQRLLPVLCQAHGLTPQQVVAIASNGGGKQALETVQRLLPVLCQAHGLTPQQVVAIASNGGGKQALETVQRLLPVLCQAHGLTPQQVVAIASHDGGKQALETVQRLLPVLCQAHGLTPQQVVAIASNIGGKQALETVQRLLPVLCQAHGLTPQQVVAIASNNGGKQALETVQRLLPVLCQAHGLTPQQVVAIASHDGGKQALETVQRLLPVLCQAHGLTPEQVVAIASHDGGKQALETVQRLLPVLCQAHGLTPQQVVAIASHDGGKQALETVQRLLPVLCQAHGLTPEQVVAIASNNGGKQALETVQALLPVLCQAHGLTPQQVVAIASNNGGKQALETVQRLLPVLCQAHGLTPEQVVAIASNGGGRPALESIVAQLSRPDPALAALTNDHLVALACLGGRPALDAVKKGLGDPISRSQLVKSELEEKKSELRHKLKYVPHEYIELIEIARNSTQDRILEMKVMEFFMKVYGYRGKHLGGSRKPDGAIYTVGSPIDYGVIVDTKAYSGGYNLPIGQADEMQRYVEENQTRNKHINPNEWWKVYPSSVTEFKFLFVSGHFKGNYKAQLTRLNHITNCNGAVLSVEELLIGGEMIKAGTLTLEEVRRKFNNGEINFAAD

SEQ ID NO: 6 - protein, 942 aa, artificial sequence
  CD38-1_Right  TALEN
MGDPKKKRKVIDKETAAAKFERQHMDSIDIADLRTLGYSQQQQEKIKPKVRSTVAQHHEALVGHGFTHAHIVALSQHPAALGTVAVKYQDMIAALPEATHEAIVGVGKQWSGARALEALLTVAGELRGPPLQLDTGQLLKIAKRGGVTAVEAVHAWRNALTGAPLNLTPQQVVAIASNGGGKQALETVQRLLPVLCQAHGLTPQQVVAIASNNGGKQALETVQRLLPVLCQAHGLTPEQVVAIASHDGGKQALETVQRLLPVLCQAHGLTPEQVVAIASNGGGKQALETVQRLLPVLCQAHGLTPEQVVAIASNNGGKQALETVQRLLPVLCQAHGLTPEQVVAIASHDGGKQALETVQRLLPVLCQAHGLTPQQVVAIASHDGGKQALETVQRLLPVLCQAHGLTPEQVVAIASNNGGKQALETVQRLLPVLCQAHGLTPEQVVAIASNNGGKQALETVQALLPVLCQAHGLTPQQVVAIASHDGGKQALETVQRLLPVLCQAHGLTPQQVVAIASNGGGKQALETVQRLLPVLCQAHGLTPQQVVAIASHDGGKQALETVQRLLPVLCQAHGLTPEQVVAIASNGGGKQALETVQRLLPVLCQAHGLTPEQVVAIASHDGGKQALETVQRLLPVLCQAHGLTPEQVVAIASNGGGKQALETVQRLLPVLCQAHGLTPQQVVAIASNIGGRPALESIVAQLSRPDPALAALTNDHLVALACLGGRPALDAVKKGLGDPISRSQLVKSELEEKKSELRHKLKYVPHEYIELIEIARNSTQDRILEMKVMEFFMKVYGYRGKHLGGSRKPDGAIYTVGSPIDYGVIVDTKAYSGGYNLPIGQADEMQRYVEENQTRNKHINPNEWWKVYPSSVTEFKFLFVSGHFKGNYKAQLTRLNHITNCNGAVLSVEELLIGGEMIKAGTLTLEEVRRKFNNGEINFAAD

SEQ ID NO: 7 - protein, 49 aa, homo sapiens
  CD38-2_TALEN target
TGATCCTCGTCGTGGTGCTCGCGGTGGTCGTCCCGAGGTGGCGCCAGCA

SEQ ID NO: 8 - protein, 936 aa, artificial sequence
  CD38-2 Left TALEN
MGDPKKKRKVIDYPYDVPDYAIDIADLRTLGYSQQQQEKIKPKVRSTVAQHHEALVGHGFTHAHIVALSQHPAALGTVAVKYQDMIAALPEATHEAIVGVGKQWSGARALEALLTVAGELRGPPLQLDTGQLLKIAKRGGVTAVEAVHAWRNALTGAPLNLTPQQVVAIASNGGGKQALETVQRLLPVLCQAHGLTPEQVVAIASNNGGKQALETVQALLPVLCQAHGLTPQQVVAIASNIGGKQALETVQRLLPVLCQAHGLTPQQVVAIASNGGGKQALETVQRLLPVLCQAHGLTPQQVVAIASHDGGKQALETVQRLLPVLCQAHGLTPQQVVAIASHDGGKQALETVQRLLPVLCQAHGLTPQQVVAIASNGGGKQALETVQRLLPVLCQAHGLTPQQVVAIASHDGGKQALETVQRLLPVLCQAHGLTPQQVVAIASNNGGKQALETVQRLLPVLCQAHGLTPQQVVAIASNGGGKQALETVQRLLPVLCQAHGLTPQQVVAIASHDGGKQALETVQRLLPVLCQAHGLTPQQVVAIASNNGGKQALETVQRLLPVLCQAHGLTPEQVVAIASNGGGKQALETVQRLLPVLCQAHGLTPQQVVAIASNNGGKQALETVQRLLPVLCQAHGLTPEQVVAIASNNGGKQALETVQALLPVLCQAHGLTPQQVVAIASNGGGRPALESIVAQLSRPDPALAALTNDHLVALACLGGRPALDAVKKGLGDPISRSQLVKSELEEKKSELRHKLKYVPHEYIELIEIARNSTQDRILEMKVMEFFMKVYGYRGKHLGGSRKPDGAIYTVGSPIDYGVIVDTKAYSGGYNLPIGQADEMQRYVEENQTRNKHINPNEWWKVYPSSVTEFKFLFVSGHFKGNYKAQLTRLNHITNCNGAVLSVEELLIGGEMIKAGTLTLEEVRRKFNNGEINFAAD

SEQ ID NO: 9 - protein, 942 aa, artificial sequence
  CD38-2 Right TALEN
MGDPKKKRKVIDKETAAAKFERQHMDSIDIADLRTLGYSQQQQEKIKPKVRSTVAQHHEALVGHGFTHAHIVALSQHPAALGTVAVKYQDMIAALPEATHEAIVGVGKQWSGARALEALLTVAGELRGPPLQLDTGQLLKIAKRGGVTAVEAVHAWRNALTGAPLNLTPQQVVAIASHDGGKQALETVQRLLPVLCQAHGLTPQQVVAIASNNGGKQALETVQRLLPVLCQAHGLTPEQVVAIASNIGGKQALETVQRLLPVLCQAHGLTPEQVVAIASNNGGKQALETVQRLLPVLCQAHGLTPEQVVAIASNNGGKQALETVQRLLPVLCQAHGLTPEQVVAIASNGGGKQALETVQRLLPVLCQAHGLTPQQVVAIASNNGGKQALETVQRLLPVLCQAHGLTPEQVVAIASNNGGKQALETVQRLLPVLCQAHGLTPEQVVAIASHDGGKQALETVQALLPVLCQAHGLTPQQVVAIASNNGGKQALETVQRLLPVLCQAHGLTPQQVVAIASHDGGKQALETVQRLLPVLCQAHGLTPQQVVAIASHDGGKQALETVQRLLPVLCQAHGLTPEQVVAIASNIGGKQALETVQRLLPVLCQAHGLTPEQVVAIASNNGGKQALETVQRLLPVLCQAHGLTPEQVVAIASHDGGKQALETVQRLLPVLCQAHGLTPQQVVAIASNIGGRPALESIVAQLSRPDPALAALTNDHLVALACLGGRPALDAVKKGLGDPISRSQLVKSELEEKKSELRHKLKYVPHEYIELIEIARNSTQDRILEMKVMEFFMKVYGYRGKHLGGSRKPDGAIYTVGSPIDYGVIVDTKAYSGGYNLPIGQADEMQRYVEENQTRNKHINPNEWWKVYPSSVTEFKFLFVSGHFKGNYKAQLTRLNHITNCNGAVLSVEELLIGGEMIKAGTLTLEEVRRKFNNGEINFAAD

SEQ ID NO: 10 - protein, 113 aa, artificial sequence
  VL chain for 25A10
DIVMTQSPSSLTVTAGEKVTMSCKSSQSLLHSGNQRNYLTWYQQKPGQPPKLLIYWASTRESGVPDRFTGSGSGTDFTLTISSVQAEDLAVYYCQNDYDYPYTFGGGTKLEIK

SEQ ID NO: 11 - protein, 12 aa, artificial sequence
  CDR1 of VL chain for 25A10
QSLLHSGNQRNY

SEQ ID NO: 12 - protein, 3 aa, artificial sequence
  CDR2 of VL chain for 25A10
WAS

SEQ ID NO: 13 - protein, 9 aa, artificial sequence
  CDR3 of VL chain for 25A10
QNDYDYPYT

SEQ ID NO: 14 - protein, 118 aa, artificial sequence
  VH chain for 25A10
EVQLQQSGAELVRPGASVKLSCTASGFNIKDSLIHWVKQRPEQGLEWIGWIDPEDDKTKYAPKFQDKATLTADTSSNTAYLQLSTLTSEDTAIYYCVSRYINYYFAYWGQGTTLTVSS

SEQ ID NO: 15 - protein, 8 aa, artificial sequence
  CDR1 of VH chain for 25A10
GFNIKDSL

SEQ ID NO: 16 - protein, 8 aa, artificial sequence
  CDR2 of VH chain for 25A10
IDPEDDKT

SEQ ID NO: 17 - protein, 11 aa, artificial sequence
  CDR3 of VH chain for 25A10
VSRYINYYFAY

SEQ ID NO: 18 - protein, 107 aa, artificial sequence
  VL chain for 29B4
DIVMTQSHKFMSTSVGDRVNITCKASQDVNTAVAWYQQKPGQSPKLLIYWASTRHAGVPDRFTGSGSGTDYALTISSVQAEDLALYYCQQHYSTPRTFGGGTKLEIK

SEQ ID NO: 19 - protein, 6 aa, artificial sequence
  CDR1 of VL chain for 29B4
QDVNTA

SEQ ID NO: 20 - protein, 3 aa, artificial sequence
  CDR2 of VL chain for 29B4
WAS

SEQ ID NO: 21 - protein, 9 aa, artificial sequence
  CDR3 of VL chain for 29B4
QQHYSTPRT

SEQ ID NO: 22 - protein, 122 aa, artificial sequence
  VH chain for 29B4
EVQLVESGGGLVKPGGSLKLSCAASGFTFSDYFMYWVRQTPEKRLEWVAIISDGGIYTYYPDSVKGRFTISRDNAKNNLYLQMSSLKSEDTAMYYCARDGRDDYDGWYFDVWGAGTTVTVSS

SEQ ID NO: 23 - protein, 8 aa, artificial sequence
  CDR1 of VH chain for 29B4
GFTFSDYF

SEQ ID NO: 24 - protein, 8 aa, artificial sequence
  CDR2 of VH chain for 29B4
ISDGGIYT

SEQ ID NO: 25 - protein, 15 aa, artificial sequence
  CDR3 of VH chain for 29B4
ARDGRDDYDGWYFDV

SEQ ID NO: 26 - protein, 111 aa, artificial sequence
  VL chain for 16B5
NIVLTQSPASLAVSLGQRATISCRASESVDNYGTTFMYWYQQKPGQPPKLLIYLASNLESGVPARFSGSGSGTDFTLTIDPVEADDAATYYCQQNKEDPWTFGGGTKLEIK

SEQ ID NO: 27 - protein, 10 aa, artificial sequence
  CDR1 of VL chain for 16B5
ESVDNYGTTF

SEQ ID NO: 28 - protein, 3 aa, artificial sequence
  CDR2 of VL chain for 16B5
LAS

SEQ ID NO: 29 - protein, 9 aa, artificial sequence
  CDR3 of VL chain for 16B5
QQNKEDPWT

SEQ ID NO: 30 - protein, 121 aa, artificial sequence
  VH chain for 16B5
QAYLQQSGAELVRSGASVKMSCKASGYTFTSYNLHWVKQTPGQGLEWIGYIYPGNGGTNYNQKFKGKATLTADTSSSTAYMQISSLTSEDSAVYFCARGGIYYYGSSLDYWGQGTTLTVSS

SEQ ID NO: 31 - protein, 8 aa, artificial sequence
  CDR1 of VH chain for 16B5
GYTFTSYN

SEQ ID NO: 32 - protein, 8 aa, artificial sequence
  CDR2 of VH chain for 16B5
IYPGNGGT

SEQ ID NO: 33 - protein, 14 aa, artificial sequence
  CDR3 of VH chain for 16B5
ARGGIYYYGSSLDY

SEQ ID NO: 34 - protein, 111 aa, artificial sequence
  VL chain for 10F7
NIVLTQSPASLAASPGQRATISCRASESVDSYGNTFMYWYQQKPGQPPKLLIYLASNLESGVPVRFSGSGSRTDFTLTIDPVEADDAATYYCQQNNEDPWTFGGGTKVEIK

SEQ ID NO: 35 - protein, 10 aa, artificial sequence
  CDR1 of VL chain for 10F7
ESVDSYGNTF

SEQ ID NO: 36 - protein, 3 aa, artificial sequence
  CDR2 of VL chain for 10F7
LAS

SEQ ID NO: 37 - protein, 9 aa, artificial sequence
  CDR3 of VL chain for 10F7
QQNNEDPWT

SEQ ID NO: 38 - protein, 120 aa, artificial sequence
  VH chain for 10F7
QAYLQQSGAELVRSGASVKMSCKASGYTFTSYNMHWVKQTPGQGLEWIGYIYPGNGGTNYNQKFKDKATLTADTSSSTAYMQISSLTSEDSAVYFCARGGQLGRPWFAYWGQGTLVTVSA

SEQ ID NO: 39 - protein, 8 aa, artificial sequence
  CDR1 of VH chain for 10F7
GYTFTSYN

SEQ ID NO: 40 - protein, 8 aa, artificial sequence
  CDR2 of VH chain for 10F7
IYPGNGGT

SEQ ID NO: 41 - protein, 13 aa, artificial sequence
  CDR3 of VH chain for 10F7
ARGGQLGRPWFAY

SEQ ID NO: 42 - protein, 106 aa, artificial sequence
  VL chain for 27B6
QIVLTQSPAIMSASPGEKVTMTCSTSSSVSYMHWYQQKSGTSPKRWIYDTSKLASGVPARFSGSGSGTSYSLTINNMEAEDAATYSCQQWSSYPPTFGGGTKLEIK

SEQ ID NO: 43 - protein, 5 aa, artificial sequence
  CDR1 of VL chain for 27B6
SSVSY

SEQ ID NO: 44 - protein, 3 aa, artificial sequence
  CDR2 of VL chain for 27B6
DTS

SEQ ID NO: 45 - protein, 9 aa, artificial sequence
  CDR3 of VL chain for 27B6
QQWSSYPPT

SEQ ID NO: 46 - protein, 122 aa, artificial sequence
  VH chain for 27B6
QVQLKQSGPGLVQPSQSLSITCTVSGFSLTSYNIDWVRQSPGKGLEWLGVIWSGGSTDYNAAFISRLKISKDDSKSQVFFKMNSLQSDDTAIYYCARHSPLVSTPDWYFDVWGAGTTVTVSS

SEQ ID NO: 47 - protein, 8 aa, artificial sequence
  CDR1 of VH chain for 27B6
GFSLTSYN

SEQ ID NO: 48 - protein, 7 aa, artificial sequence
  CDR2 of VH chain for 27B6
IWSGGST

SEQ ID NO: 49 - protein, 16 aa, artificial sequence
  CDR3 of VH chain for 27B6
ARHSPLVSTPDWYFDV

SEQ ID NO: 50 - protein, 107 aa, artificial sequence
  VL chain for 13F11
ETTVTQSPASLSVATGEKVTIRCITSTDIDDDMNWYQQKPGEPPKVLISEGNTLRPGVPSRFSSSGYGTDFVFTIENTLSEDVADYYCLQSNNMPYTFGGGTKLEIK

SEQ ID NO: 51 - protein, 6 aa, artificial sequence
  CDR1 of VL chain for 13F11
TDIDDD

SEQ ID NO: 52 - protein, 3 aa, artificial sequence
  CDR2 of VL chain for 13F11
EGN

SEQ ID NO: 53 - protein, 9 aa, artificial sequence
  CDR3 of VL chain for 13F11
LQSNNMPYT

SEQ ID NO: 54 - protein, 123 aa, artificial sequence
  VH chain for 13F11
QIQLVQSGPELKKPGETVKISCKASGYTFKKYGMNWVKQAPGKGLKWMGWINTNTGEPTYAEEFKGRFAFSLETSASTAYLQINNLKNEDTATYFCARWYYGSTPSSYTMDYWGQGTSVTVSS

SEQ ID NO: 55 - protein, 8 aa, artificial sequence
  CDR1 of VH chain for 13F11
GYTFKKYG

SEQ ID NO: 56 - protein, 8 aa, artificial sequence
  CDR2 of VH chain for 13F11
INTNTGEP

SEQ ID NO: 57 - protein, 16 aa, artificial sequence
  CDR3 of VH chain for 13F11
ARWYYGSTPSSYTMDY

SEQ ID NO: 58 - protein, 108 aa, artificial sequence
  VL chain for 28F5
QIILTQSPAIMSASLGERVTMTCTATSSLSSSYLHWYQQKPGSSPKLWIYSTSHLASGVPARFSGGGSGTSYSLTISSMEAEDAATYYCHQYHLSPYTFGGGTKLEIK

SEQ ID NO: 59 - protein, 7 aa, artificial sequence
  CDR1 of VL chain for 28F5
SSLSSSY

SEQ ID NO: 60 - protein, 3 aa, artificial sequence
  CDR2 of VL chain for 28F5
STS

SEQ ID NO: 61 - protein, 9 aa, artificial sequence
  CDR3 of VL chain for 28F5
HQYHLSPYT

SEQ ID NO: 62 - protein, 126 aa, artificial sequence
  VH chain for 28F5
QIQLVQSGPELKKPGETVKISCKASGYTFTKYGMNWVKQTPGKGLKWMGWINTNSGEPTYAEEFKGRFAFSLETSASTAYLQINNLKNEDTATYFCARGAYYRYDGEVSYYAMDYWGQGTSVTVSS

SEQ ID NO: 63 - protein, 8 aa, artificial sequence
  CDR1 of VH chain for 28F5
GYTFTKYG

SEQ ID NO: 64 - protein, 8 aa, artificial sequence
  CDR2 of VH chain for 28F5
INTNSGEP

SEQ ID NO: 65 - protein, 19 aa, artificial sequence
  CDR3 of VH chain for 28F5
ARGAYYRYDGEVSYYAMDY

SEQ ID NO: 66 - protein, 107 aa, artificial sequence [sequence omitted]

SEQ ID NO: 67 - protein, 6 aa, artificial sequence
  CDR1 of VL chain for GMB005
QSVSSY

SEQ ID NO: 68 - protein, 3 aa, artificial sequence
  CDR2 of VL chain for GMB005
DAS

SEQ ID NO: 69 - protein, 9 aa, artificial sequence
  CDR3 of VL chain for GMB005
QQRSNWPPT

SEQ ID NO: 70 - protein, 124 aa, artificial sequence
  VH chain for GMB005
EVQLLESGGGLVQPGGSLRLSCAVSGFTFNSFAMSWVRQAPGKGLEWVSAISGSGGGTYYADSVKGRFTISRDNSKNTLYLQMNSLRAEDTAVYFCAKDKILWFGEPVFDYWGQGTLVTVSSAS

SEQ ID NO: 71 - protein, 8 aa, artificial sequence
  CDR1 of VH chain for GMB005
GFTFNSFA

SEQ ID NO: 72 - protein, 8 aa, artificial sequence
  CDR2 of VH chain for GMB005
ISGSGGGT

SEQ ID NO: 73 - protein, 15 aa, artificial sequence
  CDR3 of VH chain for GMB005
AKDKILWFGEPVFDY

SEQ ID NO: 74 - protein, 21 aa, artificial sequence
  CD8a;-Signal peptide (SP)
MALPVTALLLPLALLLHAARP

SEQ ID NO: 75 - protein, 15 aa, artificial sequence
  GS linker
GGGGSGGGGSGGGGS

SEQ ID NO: 76 - protein, 16 aa, homo sapiens
  FCRIIIa; hinge
GLAVSTISSFFPPGYQ

SEQ ID NO: 77 - protein, 45 aa, homo sapiens
  CD8a; hinge
TTTPAPRPPTPAPTIASQPLSLRPEACRPAAGGAVHTRGLDFACD

SEQ ID NO: 78 - protein, 231 aa, homo sapiens
  IgG1 hinge
EPKSPDKTHTCPPCPAPPVAGPSVFLFPPKPKDTLMIARTPEVTCVVVDVSHEDPEVKFNWYVDGVEVHNAKTKPREEQYNSTYRVVSVLTVLHQDWLNGKEYKCKVSNKALPAPIEKTISKAKGQPREPQVYTLPPSRDELTKNQVSLTCLVKGFYPSDIAVEWESNGQPENNYKTTPPVLDSDGSFFLYSKLTVDKSRWQQGNVFSCSVMHEALHNHYTQKSLSLSPGK

SEQ ID NO: 79 - protein, 24 aa, homo sapiens
  CD8a; TM domain
IYIWAPLAGTCGVLLLSLVITLYC

SEQ ID NO: 80 - protein, 42 aa, homo sapiens
  4-1 BB co-stimulatory domain
KRGRKKLLYIFKQPFMRPVQTTQEEDGCSCRFPEEEEGGCEL

SEQ ID NO: 81 - protein, 112 aa, homo sapiens
  CD3&#950; activation domain
RVKFSRSADAPAYQQGQNQLYNELNLGRREEYDVLDKRRGRDPEMGGKPRRKNPQEGLYNELQKDKMAEAYSEIGMKGERRRGKGHDGLYQGLSTATKDTYDALHMQALPPR

SEQ ID NO: 82 - protein, 461 aa, artificial sequence
  25A10-V1 CAR
MALPVTALLLPLALLLHAARPEVQLQQSGAELVRPGASVKLSCTASGFNIKDSLIHWVKQRPEQGLEWIGWIDPEDDKTKYAPKFQDKATLTADTSSNTAYLQLSTLTSEDTAIYYCVSRYINYYFAYWGQGTTLTVSSGGGGSGGGGSGGGGSDIVMTQSPSSLTVTAGEKVTMSCKSSQSLLHSGNQRNYLTWYQQKPGQPPKLLIYWASTRESGVPDRFTGSGSGTDFTLTISSVQAEDLAVYYCQNDYDYPYTFGGGTKLEIKGLAVSTISSFFPPGYQIYIWAPLAGTCGVLLLSLVITLYCKRGRKKLLYIFKQPFMRPVQTTQEEDGCSCRFPEEEEGGCELRVKFSRSADAPAYQQGQNQLYNELNLGRREEYDVLDKRRGRDPEMGGKPRRKNPQEGLYNELQKDKMAEAYSEIGMKGERRRGKGHDGLYQGLSTATKDTYDALHMQALPPR

SEQ ID NO: 83 - protein, 490 aa, artificial sequence
  25A10-V2 CAR
MALPVTALLLPLALLLHAARPEVQLQQSGAELVRPGASVKLSCTASGFNIKDSLIHWVKQRPEQGLEWIGWIDPEDDKTKYAPKFQDKATLTADTSSNTAYLQLSTLTSEDTAIYYCVSRYINYYFAYWGQGTTLTVSSGGGGSGGGGSGGGGSDIVMTQSPSSLTVTAGEKVTMSCKSSQSLLHSGNQRNYLTWYQQKPGQPPKLLIYWASTRESGVPDRFTGSGSGTDFTLTISSVQAEDLAVYYCQNDYDYPYTFGGGTKLEIKTTTPAPRPPTPAPTIASQPLSLRPEACRPAAGGAVHTRGLDFACDIYIWAPLAGTCGVLLLSLVITLYCKRGRKKLLYIFKQPFMRPVQTTQEEDGCSCRFPEEEEGGCELRVKFSRSADAPAYQQGQNQLYNELNLGRREEYDVLDKRRGRDPEMGGKPRRKNPQEGLYNELQKDKMAEAYSEIGMKGERRRGKGHDGLYQGLSTATKDTYDALHMQALPPR

SEQ ID NO: 84 - protein, 676 aa, artificial sequence
  25A10-V3 CAR
MALPVTALLLPLALLLHAARPEVQLQQSGAELVRPGASVKLSCTASGFNIKDSLIHWVKQRPEQGLEWIGWIDPEDDKTKYAPKFQDKATLTADTSSNTAYLQLSTLTSEDTAIYYCVSRYINYYFAYWGQGTTLTVSSGGGGSGGGGSGGGGSDIVMTQSPSSLTVTAGEKVTMSCKSSQSLLHSGNQRNYLTWYQQKPGQPPKLLIYWASTRESGVPDRFTGSGSGTDFTLTISSVQAEDLAVYYCQNDYDYPYTFGGGTKLEIKEPKSPDKTHTCPPCPAPPVAGPSVFLFPPKPKDTLMIARTPEVTCVVVDVSHEDPEVKFNWYVDGVEVHNAKTKPREEQYNSTYRVVSVLTVLHQDWLNGKEYKCKVSNKALPAPIEKTISKAKGQPREPQVYTLPPSRDELTKNQVSLTCLVKGFYPSDIAVEWESNGQPENNYKTTPPVLDSDGSFFLYSKLTVDKSRWQQGNVFSCSVMHEALHNHYTQKSLSLSPGKIYIWAPLAGTCGVLLLSLVITLYCKRGRKKLLYIFKQPFMRPVQTTQEEDGCSCRFPEEEEGGCELRVKFSRSADAPAYQQGQNQLYNELNLGRREEYDVLDKRRGRDPEMGGKPRRKNPQEGLYNELQKDKMAEAYSEIGMKGERRRGKGHDGLYQGLSTATKDTYDALHMQALPPR

SEQ ID NO: 85 - protein, 459 aa, artificial sequence
  29B4-V1 CAR
MALPVTALLLPLALLLHAARPEVQLVESGGGLVKPGGSLKLSCAASGFTFSDYFMYWVRQTPEKRLEWVAIISDGGIYTYYPDSVKGRFTISRDNAKNNLYLQMSSLKSEDTAMYYCARDGRDDYDGWYFDVWGAGTTVTVSSGGGGSGGGGSGGGGSDIVMTQSHKFMSTSVGDRVNITCKASQDVNTAVAWYQQKPGQSPKLLIYWASTRHAGVPDRFTGSGSGTDYALTISSVQAEDLALYYCQQHYSTPRTFGGGTKLEIKGLAVSTISSFFPPGYQIYIWAPLAGTCGVLLLSLVITLYCKRGRKKLLYIFKQPFMRPVQTTQEEDGCSCRFPEEEEGGCELRVKFSRSADAPAYQQGQNQLYNELNLGRREEYDVLDKRRGRDPEMGGKPRRKNPQEGLYNELQKDKMAEAYSEIGMKGERRRGKGHDGLYQGLSTATKDTYDALHMQALPPR

SEQ ID NO: 86 - protein, 488 aa, artificial sequence
  29B4-V2 CAR
MALPVTALLLPLALLLHAARPEVQLVESGGGLVKPGGSLKLSCAASGFTFSDYFMYWVRQTPEKRLEWVAIISDGGIYTYYPDSVKGRFTISRDNAKNNLYLQMSSLKSEDTAMYYCARDGRDDYDGWYFDVWGAGTTVTVSSGGGGSGGGGSGGGGSDIVMTQSHKFMSTSVGDRVNITCKASQDVNTAVAWYQQKPGQSPKLLIYWASTRHAGVPDRFTGSGSGTDYALTISSVQAEDLALYYCQQHYSTPRTFGGGTKLEIKTTTPAPRPPTPAPTIASQPLSLRPEACRPAAGGAVHTRGLDFACDIYIWAPLAGTCGVLLLSLVITLYCKRGRKKLLYIFKQPFMRPVQTTQEEDGCSCRFPEEEEGGCELRVKFSRSADAPAYQQGQNQLYNELNLGRREEYDVLDKRRGRDPEMGGKPRRKNPQEGLYNELQKDKMAEAYSEIGMKGERRRGKGHDGLYQGLSTATKDTYDALHMQALPPR

SEQ ID NO: 87 - protein, 674 aa, artificial sequence
  29B4-V3 CAR
MALPVTALLLPLALLLHAARPEVQLVESGGGLVKPGGSLKLSCAASGFTFSDYFMYWVRQTPEKRLEWVAIISDGGIYTYYPDSVKGRFTISRDNAKNNLYLQMSSLKSEDTAMYYCARDGRDDYDGWYFDVWGAGTTVTVSSGGGGSGGGGSGGGGSDIVMTQSHKFMSTSVGDRVNITCKASQDVNTAVAWYQQKPGQSPKLLIYWASTRHAGVPDRFTGSGSGTDYALTISSVQAEDLALYYCQQHYSTPRTFGGGTKLEIKEPKSPDKTHTCPPCPAPPVAGPSVFLFPPKPKDTLMIARTPEVTCVVVDVSHEDPEVKFNWYVDGVEVHNAKTKPREEQYNSTYRVVSVLTVLHQDWLNGKEYKCKVSNKALPAPIEKTISKAKGQPREPQVYTLPPSRDELTKNQVSLTCLVKGFYPSDIAVEWESNGQPENNYKTTPPVLDSDGSFFLYSKLTVDKSRWQQGNVFSCSVMHEALHNHYTQKSLSLSPGKIYIWAPLAGTCGVLLLSLVITLYCKRGRKKLLYIFKQPFMRPVQTTQEEDGCSCRFPEEEEGGCELRVKFSRSADAPAYQQGQNQLYNELNLGRREEYDVLDKRRGRDPEMGGKPRRKNPQEGLYNELQKDKMAEAYSEIGMKGERRRGKGHDGLYQGLSTATKDTYDALHMQALPPR

SEQ ID NO: 88 - protein, 462 aa, artificial sequence
  16B5-V1 CAR
MALPVTALLLPLALLLHAARPQAYLQQSGAELVRSGASVKMSCKASGYTFTSYNLHWVKQTPGQGLEWIGYIYPGNGGTNYNQKFKGKATLTADTSSSTAYMQISSLTSEDSAVYFCARGGIYYYGSSLDYWGQGTTLTVSSGGGGSGGGGSGGGGSNIVLTQSPASLAVSLGQRATISCRASESVDNYGTTFMYWYQQKPGQPPKLLIYLASNLESGVPARFSGSGSGTDFTLTIDPVEADDAATYYCQQNKEDPWTFGGGTKLEIKGLAVSTISSFFPPGYQIYIWAPLAGTCGVLLLSLVITLYCKRGRKKLLYIFKQPFMRPVQTTQEEDGCSCRFPEEEEGGCELRVKFSRSADAPAYQQGQNQLYNELNLGRREEYDVLDKRRGRDPEMGGKPRRKNPQEGLYNELQKDKMAEAYSEIGMKGERRRGKGHDGLYQGLSTATKDTYDALHMQALPPR

SEQ ID NO: 89 - protein, 491 aa, artificial sequence
  16B5-V2 CAR
MALPVTALLLPLALLLHAARPQAYLQQSGAELVRSGASVKMSCKASGYTFTSYNLHWVKQTPGQGLEWIGYIYPGNGGTNYNQKFKGKATLTADTSSSTAYMQISSLTSEDSAVYFCARGGIYYYGSSLDYWGQGTTLTVSSGGGGSGGGGSGGGGSNIVLTQSPASLAVSLGQRATISCRASESVDNYGTTFMYWYQQKPGQPPKLLIYLASNLESGVPARFSGSGSGTDFTLTIDPVEADDAATYYCQQNKEDPWTFGGGTKLEIKTTTPAPRPPTPAPTIASQPLSLRPEACRPAAGGAVHTRGLDFACDIYIWAPLAGTCGVLLLSLVITLYCKRGRKKLLYIFKQPFMRPVQTTQEEDGCSCRFPEEEEGGCELRVKFSRSADAPAYQQGQNQLYNELNLGRREEYDVLDKRRGRDPEMGGKPRRKNPQEGLYNELQKDKMAEAYSEIGMKGERRRGKGHDGLYQGLSTATKDTYDALHMQALPPR

SEQ ID NO: 90 - protein, 677 aa, artificial sequence
  16B5-V3 CAR
MALPVTALLLPLALLLHAARPQAYLQQSGAELVRSGASVKMSCKASGYTFTSYNLHWVKQTPGQGLEWIGYIYPGNGGTNYNQKFKGKATLTADTSSSTAYMQISSLTSEDSAVYFCARGGIYYYGSSLDYWGQGTTLTVSSGGGGSGGGGSGGGGSNIVLTQSPASLAVSLGQRATISCRASESVDNYGTTFMYWYQQKPGQPPKLLIYLASNLESGVPARFSGSGSGTDFTLTIDPVEADDAATYYCQQNKEDPWTFGGGTKLEIKEPKSPDKTHTCPPCPAPPVAGPSVFLFPPKPKDTLMIARTPEVTCVVVDVSHEDPEVKFNWYVDGVEVHNAKTKPREEQYNSTYRVVSVLTVLHQDWLNGKEYKCKVSNKALPAPIEKTISKAKGQPREPQVYTLPPSRDELTKNQVSLTCLVKGFYPSDIAVEWESNGQPENNYKTTPPVLDSDGSFFLYSKLTVDKSRWQQGNVFSCSVMHEALHNHYTQKSLSLSPGKIYIWAPLAGTCGVLLLSLVITLYCKRGRKKLLYIFKQPFMRPVQTTQEEDGCSCRFPEEEEGGCELRVKFSRSADAPAYQQGQNQLYNELNLGRREEYDVLDKRRGRDPEMGGKPRRKNPQEGLYNELQKDKMAEAYSEIGMKGERRRGKGHDGLYQGLSTATKDTYDALHMQALPPR

SEQ ID NO: 91 - protein, 461 aa, artificial sequence
  10F7-V1 CAR
MALPVTALLLPLALLLHAARPQAYLQQSGAELVRSGASVKMSCKASGYTFTSYNMHWVKQTPGQGLEWIGYIYPGNGGTNYNQKFKDKATLTADTSSSTAYMQISSLTSEDSAVYFCARGGQLGRPWFAYWGQGTLVTVSAGGGGSGGGGSGGGGSNIVLTQSPASLAASPGQRATISCRASESVDSYGNTFMYWYQQKPGQPPKLLIYLASNLESGVPVRFSGSGSRTDFTLTIDPVEADDAATYYCQQNNEDPWTFGGGTKVEIKGLAVSTISSFFPPGYQIYIWAPLAGTCGVLLLSLVITLYCKRGRKKLLYIFKQPFMRPVQTTQEEDGCSCRFPEEEEGGCELRVKFSRSADAPAYQQGQNQLYNELNLGRREEYDVLDKRRGRDPEMGGKPRRKNPQEGLYNELQKDKMAEAYSEIGMKGERRRGKGHDGLYQGLSTATKDTYDALHMQALPPR

SEQ ID NO: 92 - protein, 490 aa, artificial sequence
  10F7-V2 CAR
MALPVTALLLPLALLLHAARPQAYLQQSGAELVRSGASVKMSCKASGYTFTSYNMHWVKQTPGQGLEWIGYIYPGNGGTNYNQKFKDKATLTADTSSSTAYMQISSLTSEDSAVYFCARGGQLGRPWFAYWGQGTLVTVSAGGGGSGGGGSGGGGSNIVLTQSPASLAASPGQRATISCRASESVDSYGNTFMYWYQQKPGQPPKLLIYLASNLESGVPVRFSGSGSRTDFTLTIDPVEADDAATYYCQQNNEDPWTFGGGTKVEIKTTTPAPRPPTPAPTIASQPLSLRPEACRPAAGGAVHTRGLDFACDIYIWAPLAGTCGVLLLSLVITLYCKRGRKKLLYIFKQPFMRPVQTTQEEDGCSCRFPEEEEGGCELRVKFSRSADAPAYQQGQNQLYNELNLGRREEYDVLDKRRGRDPEMGGKPRRKNPQEGLYNELQKDKMAEAYSEIGMKGERRRGKGHDGLYQGLSTATKDTYDALHMQALPPR

SEQ ID NO: 93 - protein, 676 aa, artificial sequence
  10F7-V3 CAR
MALPVTALLLPLALLLHAARPQAYLQQSGAELVRSGASVKMSCKASGYTFTSYNMHWVKQTPGQGLEWIGYIYPGNGGTNYNQKFKDKATLTADTSSSTAYMQISSLTSEDSAVYFCARGGQLGRPWFAYWGQGTLVTVSAGGGGSGGGGSGGGGSNIVLTQSPASLAASPGQRATISCRASESVDSYGNTFMYWYQQKPGQPPKLLIYLASNLESGVPVRFSGSGSRTDFTLTIDPVEADDAATYYCQQNNEDPWTFGGGTKVEIKEPKSPDKTHTCPPCPAPPVAGPSVFLFPPKPKDTLMIARTPEVTCVVVDVSHEDPEVKFNWYVDGVEVHNAKTKPREEQYNSTYRVVSVLTVLHQDWLNGKEYKCKVSNKALPAPIEKTISKAKGQPREPQVYTLPPSRDELTKNQVSLTCLVKGFYPSDIAVEWESNGQPENNYKTTPPVLDSDGSFFLYSKLTVDKSRWQQGNVFSCSVMHEALHNHYTQKSLSLSPGKIYIWAPLAGTCGVLLLSLVITLYCKRGRKKLLYIFKQPFMRPVQTTQEEDGCSCRFPEEEEGGCELRVKFSRSADAPAYQQGQNQLYNELNLGRREEYDVLDKRRGRDPEMGGKPRRKNPQEGLYNELQKDKMAEAYSEIGMKGERRRGKGHDGLYQGLSTATKDTYDALHMQALPPR

SEQ ID NO: 94 - protein, 458 aa, artificial sequence
  27B6-V1 CAR
MALPVTALLLPLALLLHAARPQVQLKQSGPGLVQPSQSLSITCTVSGFSLTSYNIDWVRQSPGKGLEWLGVIWSGGSTDYNAAFISRLKISKDDSKSQVFFKMNSLQSDDTAIYYCARHSPLVSTPDWYFDVWGAGTTVTVSSGGGGSGGGGSGGGGSQIVLTQSPAIMSASPGEKVTMTCSTSSSVSYMHWYQQKSGTSPKRWIYDTSKLASGVPARFSGSGSGTSYSLTINNMEAEDAATYSCQQWSSYPPTFGGGTKLEIKGLAVSTISSFFPPGYQIYIWAPLAGTCGVLLLSLVITLYCKRGRKKLLYIFKQPFMRPVQTTQEEDGCSCRFPEEEEGGCELRVKFSRSADAPAYQQGQNQLYNELNLGRREEYDVLDKRRGRDPEMGGKPRRKNPQEGLYNELQKDKMAEAYSEIGMKGERRRGKGHDGLYQGLSTATKDTYDALHMQALPPR

SEQ ID NO: 95 - protein, 487 aa, artificial sequence
  27B6-V2 CAR
MALPVTALLLPLALLLHAARPQVQLKQSGPGLVQPSQSLSITCTVSGFSLTSYNIDWVRQSPGKGLEWLGVIWSGGSTDYNAAFISRLKISKDDSKSQVFFKMNSLQSDDTAIYYCARHSPLVSTPDWYFDVWGAGTTVTVSSGGGGSGGGGSGGGGSQIVLTQSPAIMSASPGEKVTMTCSTSSSVSYMHWYQQKSGTSPKRWIYDTSKLASGVPARFSGSGSGTSYSLTINNMEAEDAATYSCQQWSSYPPTFGGGTKLEIKTTTPAPRPPTPAPTIASQPLSLRPEACRPAAGGAVHTRGLDFACDIYIWAPLAGTCGVLLLSLVITLYCKRGRKKLLYIFKQPFMRPVQTTQEEDGCSCRFPEEEEGGCELRVKFSRSADAPAYQQGQNQLYNELNLGRREEYDVLDKRRGRDPEMGGKPRRKNPQEGLYNELQKDKMAEAYSEIGMKGERRRGKGHDGLYQGLSTATKDTYDALHMQALPPR

SEQ ID NO: 96 - protein, 673 aa, artificial sequence
  27B6-V3 CAR
MALPVTALLLPLALLLHAARPQVQLKQSGPGLVQPSQSLSITCTVSGFSLTSYNIDWVRQSPGKGLEWLGVIWSGGSTDYNAAFISRLKISKDDSKSQVFFKMNSLQSDDTAIYYCARHSPLVSTPDWYFDVWGAGTTVTVSSGGGGSGGGGSGGGGSQIVLTQSPAIMSASPGEKVTMTCSTSSSVSYMHWYQQKSGTSPKRWIYDTSKLASGVPARFSGSGSGTSYSLTINNMEAEDAATYSCQQWSSYPPTFGGGTKLEIKEPKSPDKTHTCPPCPAPPVAGPSVFLFPPKPKDTLMIARTPEVTCVVVDVSHEDPEVKFNWYVDGVEVHNAKTKPREEQYNSTYRVVSVLTVLHQDWLNGKEYKCKVSNKALPAPIEKTISKAKGQPREPQVYTLPPSRDELTKNQVSLTCLVKGFYPSDIAVEWESNGQPENNYKTTPPVLDSDGSFFLYSKLTVDKSRWQQGNVFSCSVMHEALHNHYTQKSLSLSPGKIYIWAPLAGTCGVLLLSLVITLYCKRGRKKLLYIFKQPFMRPVQTTQEEDGCSCRFPEEEEGGCELRVKFSRSADAPAYQQGQNQLYNELNLGRREEYDVLDKRRGRDPEMGGKPRRKNPQEGLYNELQKDKMAEAYSEIGMKGERRRGKGHDGLYQGLSTATKDTYDALHMQALPPR

SEQ ID NO: 97 - protein, 460 aa, artificial sequence
  13F11-V1 CAR
MALPVTALLLPLALLLHAARPQIQLVQSGPELKKPGETVKISCKASGYTFKKYGMNWVKQAPGKGLKWMGWINTNTGEPTYAEEFKGRFAFSLETSASTAYLQINNLKNEDTATYFCARWYYGSTPSSYTMDYWGQGTSVTVSSGGGGSGGGGSGGGGSETTVTQSPASLSVATGEKVTIRCITSTDIDDDMNWYQQKPGEPPKVLISEGNTLRPGVPSRFSSSGYGTDFVFTIENTLSEDVADYYCLQSNNMPYTFGGGTKLEIKGLAVSTISSFFPPGYQIYIWAPLAGTCGVLLLSLVITLYCKRGRKKLLYIFKQPFMRPVQTTQEEDGCSCRFPEEEEGGCELRVKFSRSADAPAYQQGQNQLYNELNLGRREEYDVLDKRRGRDPEMGGKPRRKNPQEGLYNELQKDKMAEAYSEIGMKGERRRGKGHDGLYQGLSTATKDTYDALHMQALPPR

SEQ ID NO: 98 - protein, 489 aa, artificial sequence
  13F11-V2 CAR
MALPVTALLLPLALLLHAARPQIQLVQSGPELKKPGETVKISCKASGYTFKKYGMNWVKQAPGKGLKWMGWINTNTGEPTYAEEFKGRFAFSLETSASTAYLQINNLKNEDTATYFCARWYYGSTPSSYTMDYWGQGTSVTVSSGGGGSGGGGSGGGGSETTVTQSPASLSVATGEKVTIRCITSTDIDDDMNWYQQKPGEPPKVLISEGNTLRPGVPSRFSSSGYGTDFVFTIENTLSEDVADYYCLQSNNMPYTFGGGTKLEIKTTTPAPRPPTPAPTIASQPLSLRPEACRPAAGGAVHTRGLDFACDIYIWAPLAGTCGVLLLSLVITLYCKRGRKKLLYIFKQPFMRPVQTTQEEDGCSCRFPEEEEGGCELRVKFSRSADAPAYQQGQNQLYNELNLGRREEYDVLDKRRGRDPEMGGKPRRKNPQEGLYNELQKDKMAEAYSEIGMKGERRRGKGHDGLYQGLSTATKDTYDALHMQALPPR

SEQ ID NO: 99 - protein, 675 aa, artificial sequence
  13F11-V3 CAR
MALPVTALLLPLALLLHAARPQIQLVQSGPELKKPGETVKISCKASGYTFKKYGMNWVKQAPGKGLKWMGWINTNTGEPTYAEEFKGRFAFSLETSASTAYLQINNLKNEDTATYFCARWYYGSTPSSYTMDYWGQGTSVTVSSGGGGSGGGGSGGGGSETTVTQSPASLSVATGEKVTIRCITSTDIDDDMNWYQQKPGEPPKVLISEGNTLRPGVPSRFSSSGYGTDFVFTIENTLSEDVADYYCLQSNNMPYTFGGGTKLEIKEPKSPDKTHTCPPCPAPPVAGPSVFLFPPKPKDTLMIARTPEVTCVVVDVSHEDPEVKFNWYVDGVEVHNAKTKPREEQYNSTYRVVSVLTVLHQDWLNGKEYKCKVSNKALPAPIEKTISKAKGQPREPQVYTLPPSRDELTKNQVSLTCLVKGFYPSDIAVEWESNGQPENNYKTTPPVLDSDGSFFLYSKLTVDKSRWQQGNVFSCSVMHEALHNHYTQKSLSLSPGKIYIWAPLAGTCGVLLLSLVITLYCKRGRKKLLYIFKQPFMRPVQTTQEEDGCSCRFPEEEEGGCELRVKFSRSADAPAYQQGQNQLYNELNLGRREEYDVLDKRRGRDPEMGGKPRRKNPQEGLYNELQKDKMAEAYSEIGMKGERRRGKGHDGLYQGLSTATKDTYDALHMQALPPR

SEQ ID NO: 100 - protein, 464 aa, artificial sequence
  28F5-V1 CAR
MALPVTALLLPLALLLHAARPQIQLVQSGPELKKPGETVKISCKASGYTFTKYGMNWVKQTPGKGLKWMGWINTNSGEPTYAEEFKGRFAFSLETSASTAYLQINNLKNEDTATYFCARGAYYRYDGEVSYYAMDYWGQGTSVTVSSGGGGSGGGGSGGGGSQIILTQSPAIMSASLGERVTMTCTATSSLSSSYLHWYQQKPGSSPKLWIYSTSHLASGVPARFSGGGSGTSYSLTISSMEAEDAATYYCHQYHLSPYTFGGGTKLEIKGLAVSTISSFFPPGYQIYIWAPLAGTCGVLLLSLVITLYCKRGRKKLLYIFKQPFMRPVQTTQEEDGCSCRFPEEEEGGCELRVKFSRSADAPAYQQGQNQLYNELNLGRREEYDVLDKRRGRDPEMGGKPRRKNPQEGLYNELQKDKMAEAYSEIGMKGERRRGKGHDGLYQGLSTATKDTYDALHMQALPPR

SEQ ID NO: 101 - protein, 493 aa, artificial sequence
  28F5-V2 CAR
MALPVTALLLPLALLLHAARPQIQLVQSGPELKKPGETVKISCKASGYTFTKYGMNWVKQTPGKGLKWMGWINTNSGEPTYAEEFKGRFAFSLETSASTAYLQINNLKNEDTATYFCARGAYYRYDGEVSYYAMDYWGQGTSVTVSSGGGGSGGGGSGGGGSQIILTQSPAIMSASLGERVTMTCTATSSLSSSYLHWYQQKPGSSPKLWIYSTSHLASGVPARFSGGGSGTSYSLTISSMEAEDAATYYCHQYHLSPYTFGGGTKLEIKTTTPAPRPPTPAPTIASQPLSLRPEACRPAAGGAVHTRGLDFACDIYIWAPLAGTCGVLLLSLVITLYCKRGRKKLLYIFKQPFMRPVQTTQEEDGCSCRFPEEEEGGCELRVKFSRSADAPAYQQGQNQLYNELNLGRREEYDVLDKRRGRDPEMGGKPRRKNPQEGLYNELQKDKMAEAYSEIGMKGERRRGKGHDGLYQGLSTATKDTYDALHMQALPPR

SEQ ID NO: 102 - protein, 679 aa, artificial sequence
  28F5-V3 CAR
MALPVTALLLPLALLLHAARPQIQLVQSGPELKKPGETVKISCKASGYTFTKYGMNWVKQTPGKGLKWMGWINTNSGEPTYAEEFKGRFAFSLETSASTAYLQINNLKNEDTATYFCARGAYYRYDGEVSYYAMDYWGQGTSVTVSSGGGGSGGGGSGGGGSQIILTQSPAIMSASLGERVTMTCTATSSLSSSYLHWYQQKPGSSPKLWIYSTSHLASGVPARFSGGGSGTSYSLTISSMEAEDAATYYCHQYHLSPYTFGGGTKLEIKEPKSPDKTHTCPPCPAPPVAGPSVFLFPPKPKDTLMIARTPEVTCVVVDVSHEDPEVKFNWYVDGVEVHNAKTKPREEQYNSTYRVVSVLTVLHQDWLNGKEYKCKVSNKALPAPIEKTISKAKGQPREPQVYTLPPSRDELTKNQVSLTCLVKGFYPSDIAVEWESNGQPENNYKTTPPVLDSDGSFFLYSKLTVDKSRWQQGNVFSCSVMHEALHNHYTQKSLSLSPGKIYIWAPLAGTCGVLLLSLVITLYCKRGRKKLLYIFKQPFMRPVQTTQEEDGCSCRFPEEEEGGCELRVKFSRSADAPAYQQGQNQLYNELNLGRREEYDVLDKRRGRDPEMGGKPRRKNPQEGLYNELQKDKMAEAYSEIGMKGERRRGKGHDGLYQGLSTATKDTYDALHMQALPPR

SEQ ID NO: 103 - protein, 461 aa, artificial sequence
  GMB005-V1 CAR
MALPVTALLLPLALLLHAARPEVQLLESGGGLVQPGGSLRLSCAVSGFTFNSFAMSWVRQAPGKGLEWVSAISGSGGGTYYADSVKGRFTISRDNSKNTLYLQMNSLRAEDTAVYFCAKDKILWFGEPVFDYWGQGTLVTVSSASGGGGSGGGGSGGGGSEIVLTQSPATLSLSPGERATLSCRASQSVSSYLAWYQQKPGQAPRLLIYDASNRATGIPARFSGSGSGTDFTLTISSLEPEDFAVYYCQQRSNWPPTFGQGTKVEIKGLAVSTISSFFPPGYQIYIWAPLAGTCGVLLLSLVITLYCKRGRKKLLYIFKQPFMRPVQTTQEEDGCSCRFPEEEEGGCELRVKFSRSADAPAYQQGQNQLYNELNLGRREEYDVLDKRRGRDPEMGGKPRRKNPQEGLYNELQKDKMAEAYSEIGMKGERRRGKGHDGLYQGLSTATKDTYDALHMQALPPR

SEQ ID NO: 104 - protein, 490 aa, artificial sequence
  GMB005-V2 CAR
MALPVTALLLPLALLLHAARPEVQLLESGGGLVQPGGSLRLSCAVSGFTFNSFAMSWVRQAPGKGLEWVSAISGSGGGTYYADSVKGRFTISRDNSKNTLYLQMNSLRAEDTAVYFCAKDKILWFGEPVFDYWGQGTLVTVSSASGGGGSGGGGSGGGGSEIVLTQSPATLSLSPGERATLSCRASQSVSSYLAWYQQKPGQAPRLLIYDASNRATGIPARFSGSGSGTDFTLTISSLEPEDFAVYYCQQRSNWPPTFGQGTKVEIKTTTPAPRPPTPAPTIASQPLSLRPEACRPAAGGAVHTRGLDFACDIYIWAPLAGTCGVLLLSLVITLYCKRGRKKLLYIFKQPFMRPVQTTQEEDGCSCRFPEEEEGGCELRVKFSRSADAPAYQQGQNQLYNELNLGRREEYDVLDKRRGRDPEMGGKPRRKNPQEGLYNELQKDKMAEAYSEIGMKGERRRGKGHDGLYQGLSTATKDTYDALHMQALPPR

SEQ ID NO: 105 - protein, 676 aa, artificial sequence
  GMB005-V3 CAR
MALPVTALLLPLALLLHAARPEVQLLESGGGLVQPGGSLRLSCAVSGFTFNSFAMSWVRQAPGKGLEWVSAISGSGGGTYYADSVKGRFTISRDNSKNTLYLQMNSLRAEDTAVYFCAKDKILWFGEPVFDYWGQGTLVTVSSASGGGGSGGGGSGGGGSEIVLTQSPATLSLSPGERATLSCRASQSVSSYLAWYQQKPGQAPRLLIYDASNRATGIPARFSGSGSGTDFTLTISSLEPEDFAVYYCQQRSNWPPTFGQGTKVEIKEPKSPDKTHTCPPCPAPPVAGPSVFLFPPKPKDTLMIARTPEVTCVVVDVSHEDPEVKFNWYVDGVEVHNAKTKPREEQYNSTYRVVSVLTVLHQDWLNGKEYKCKVSNKALPAPIEKTISKAKGQPREPQVYTLPPSRDELTKNQVSLTCLVKGFYPSDIAVEWESNGQPENNYKTTPPVLDSDGSFFLYSKLTVDKSRWQQGNVFSCSVMHEALHNHYTQKSLSLSPGKIYIWAPLAGTCGVLLLSLVITLYCKRGRKKLLYIFKQPFMRPVQTTQEEDGCSCRFPEEEEGGCELRVKFSRSADAPAYQQGQNQLYNELNLGRREEYDVLDKRRGRDPEMGGKPRRKNPQEGLYNELQKDKMAEAYSEIGMKGERRRGKGHDGLYQGLSTATKDTYDALHMQALPPR

SEQ ID NO: 106 - protein, 18 aa, homosapiens
  Fc&#949;RI &#947;- signal peptide (SP)
MIPAVVLLLLLLVEQAAA

SEQ ID NO: 107 - protein, 43 aa, homosapiens
  Fc Receptor for IgE, gamma chain, without ITAM) (Fc&#949;RI &#947; - DITAM)
LGEPQLCYILDAILFLYGIVLTLLYCRLKIQVRKAAITSYEKS

SEQ ID NO: 108 - protein, 22 aa, artificial sequence
  GSG-P2A ribosomal skip peptide (GSG-P2A)
GSGATNFSLLKQAGDVEENPGP

SEQ ID NO: 109 - protein, 21 aa, artificial sequence
  GSG-T2A ribosomal skip peptide (GSG-T2A)
GSGEGRGSLLTCGDVEENPGP

SEQ ID NO: 110 - protein, 25 aa, homosapiens
  Fc&#949;RI a- signal peptide (SP)
MAPAMESPTLLCVALLFFAPDGVLA

SEQ ID NO: 111 - protein, 52 aa, homosapiens
  Fc Receptor for IgE, alpha chain, transmembrane and intracellular domain (Fc&#949;RI a-TM-IC)
FFIPLLVVILFAVDTGLFISTQQQVTFLLKIKRTRKGFRLLNPHPKPNPKNN

SEQ ID NO: 112 - protein, 215 aa, homosapiens
  Receptor for IgE, beta chain, without ITAM (Fc&#949;R1&#947;-&#916;ITAM)
MDTESNRRANLALPQEPSSVPAFEVLEISPQEVSSGRLLKSASSPPLHTWLTVLKKEQEFLGVTQILTAMICLCFGTVVCSVLDISHIEGDIFSSFKAGYPFWGAIFFSISGMLSIISERRNATYLVRGSLGANTASSIAGGTGITILIINLKKSLAYIHIHSCQKFFETKCFMASFSTEIVVMMLFLTILGLGSAVSLTICGAGEELKGNKVPE

SEQ ID NO: 113 - protein, 41 aa, homosapiens
  CD28 co-stimulatory domain (CD28-IC)
RSKRSRGGHSDYMNMTPRRPGPTRKHYQPYAPPRDFAAYRS

SEQ ID NO: 114 - protein, 10 aa, artificial sequence
  CD20 mimotope
CPYSNPSLCS

SEQ ID NO: 115 - protein, 24 aa, artificial sequence
  Epitope for palivizumab
NSELLSLINDMPITNDQKKLMSNN

SEQ ID NO: 116 - protein, 12 aa, artificial sequence
  Mimotope 1 for cetuximab
CQFDLSTRRLKC

SEQ ID NO: 117 - protein, 12 aa, artificial sequence
  Mimotope 2 for cetuximab
CQYNLSSRALKC

SEQ ID NO: 118 - protein, 12 aa, artificial sequence
  Mimotope 3 for cetuximab
CVWQRWQKSYVC

SEQ ID NO: 119 - protein, 12 aa, artificial sequence
  Mimotope 4 for cetuximab
CMWDRFSRWYKC

SEQ ID NO: 120 - protein, 25 aa, artificial sequence
  Epitope A for nivolumab
SFVLNWYRMSPSNQTDKLAAFPEDR

SEQ ID NO: 121 - protein, 19 aa, artificial sequence
  Epitope B for nivolumab
SGTYLCGAISLAPKAQIKE

SEQ ID NO: 122 - protein, 14 aa, artificial sequence
  Epitope 1 for CD34
TFSNVSTNVSYQET

SEQ ID NO: 123 - protein, 14 aa, artificial sequence
  Epitope 2 for CD34
NTNSSVQSQTSVIS

SEQ ID NO: 124 - protein, 533 aa, artificial sequence
  28F5v2 CAR with 2 CD20 mimotopes
MALPVTALLLPLALLLHAARPQIQLVQSGPELKKPGETVKISCKASGYTFTKYGMNWVKQTPGKGLKWMGWINTNSGEPTYAEEFKGRFAFSLETSASTAYLQINNLKNEDTATYFCARGAYYRYDGEVSYYAMDYWGQGTSVTVSSGGGGSGGGGSGGGGSQIILTQSPAIMSASLGERVTMTCTATSSLSSSYLHWYQQKPGSSPKLWIYSTSHLASGVPARFSGGGSGTSYSLTISSMEAEDAATYYCHQYHLSPYTFGGGTKLEIKSDPGSGGGGSCPYSNPSLCSGGGGSCPYSNPSLCSGGGGSTTTPAPRPPTPAPTIASQPLSLRPEACRPAAGGAVHTRGLDFACDIYIWAPLAGTCGVLLLSLVITLYCKRGRKKLLYIFKQPFMRPVQTTQEEDGCSCRFPEEEEGGCELRVKFSRSADAPAYQQGQNQLYNELNLGRREEYDVLDKRRGRDPEMGGKPRRKNPQEGLYNELQKDKMAEAYSEIGMKGERRRGKGHDGLYQGLSTATKDTYDALHMQALPPR

SEQ ID NO: 125 - protein, 573 aa, artificial sequence
  28F5v2 CAR with 2 CD20 mimotopes and 1 CD34 epitope
MALPVTALLLPLALLLHAARPGGGGSCPYSNPSLCSGGGGSGGGGSQIQLVQSGPELKKPGETVKISCKASGYTFTKYGMNWVKQTPGKGLKWMGWINTNSGEPTYAEEFKGRFAFSLETSASTAYLQINNLKNEDTATYFCARGAYYRYDGEVSYYAMDYWGQGTSVTVSSGGGGSGGGGSGGGGSQIILTQSPAIMSASLGERVTMTCTATSSLSSSYLHWYQQKPGSSPKLWIYSTSHLASGVPARFSGGGSGTSYSLTISSMEAEDAATYYCHQYHLSPYTFGGGTKLEIKGSGGGGSCPYSNPSLCSGGGGSELPTQGTFSNVSTNVSPAKPTTTACPYSNPSLCTTTPAPRPPTPAPTIASQPLSLRPEACRPAAGGAVHTRGLDFACDIYIWAPLAGTCGVLLLSLVITLYCKRGRKKLLYIFKQPFMRPVQTTQEEDGCSCRFPEEEEGGCELRVKFSRSADAPAYQQGQNQLYNELNLGRREEYDVLDKRRGRDPEMGGKPRRKNPQEGLYNELQKDKMAEAYSEIGMKGERRRGKGHDGLYQGLSTATKDTYDALHMQALPPR

SEQ ID NO: 126 - protein, 504 aa, artificial sequence
  28F5v1 CAR with 2 CD20 mimotopes
MALPVTALLLPLALLLHAARPQIQLVQSGPELKKPGETVKISCKASGYTFTKYGMNWVKQTPGKGLKWMGWINTNSGEPTYAEEFKGRFAFSLETSASTAYLQINNLKNEDTATYFCARGAYYRYDGEVSYYAMDYWGQGTSVTVSSGGGGSGGGGSGGGGSQIILTQSPAIMSASLGERVTMTCTATSSLSSSYLHWYQQKPGSSPKLWIYSTSHLASGVPARFSGGGSGTSYSLTISSMEAEDAATYYCHQYHLSPYTFGGGTKLEIKSDPGSGGGGSCPYSNPSLCSGGGGSCPYSNPSLCSGGGGSGLAVSTISSFFPPGYQIYIWAPLAGTCGVLLLSLVITLYCKRGRKKLLYIFKQPFMRPVQTTQEEDGCSCRFPEEEEGGCELRVKFSRSADAPAYQQGQNQLYNELNLGRREEYDVLDKRRGRDPEMGGKPRRKNPQEGLYNELQKDKMAEAYSEIGMKGERRRGKGHDGLYQGLSTATKDTYDALHMQALPPR

SEQ ID NO: 127 - protein, 544 aa, artificial sequence
  28F5v1 CAR with 2 CD20 mimotopes and 1 CD34 epitope
MALPVTALLLPLALLLHAARPGGGGSCPYSNPSLCSGGGGSGGGGSQIQLVQSGPELKKPGETVKISCKASGYTFTKYGMNWVKQTPGKGLKWMGWINTNSGEPTYAEEFKGRFAFSLETSASTAYLQINNLKNEDTATYFCARGAYYRYDGEVSYYAMDYWGQGTSVTVSSGGGGSGGGGSGGGGSQIILTQSPAIMSASLGERVTMTCTATSSLSSSYLHWYQQKPGSSPKLWIYSTSHLASGVPARFSGGGSGTSYSLTISSMEAEDAATYYCHQYHLSPYTFGGGTKLEIKGSGGGGSCPYSNPSLCSGGGGSELPTQGTFSNVSTNVSPAKPTTTACPYSNPSLCGLAVSTISSFFPPGYQIYIWAPLAGTCGVLLLSLVITLYCKRGRKKLLYIFKQPFMRPVQTTQEEDGCSCRFPEEEEGGCELRVKFSRSADAPAYQQGQNQLYNELNLGRREEYDVLDKRRGRDPEMGGKPRRKNPQEGLYNELQKDKMAEAYSEIGMKGERRRGKGHDGLYQGLSTATKDTYDALHMQALPPR

SEQ ID NO: 128 - protein, 530 aa, artificial sequence
  25A10v2 CAR with 2 CD20 mimotopes
MALPVTALLLPLALLLHAARPEVQLQQSGAELVRPGASVKLSCTASGFNIKDSLIHWVKQRPEQGLEWIGWIDPEDDKTKYAPKFQDKATLTADTSSNTAYLQLSTLTSEDTAIYYCVSRYINYYFAYWGQGTTLTVSSGGGGSGGGGSGGGGSDIVMTQSPSSLTVTAGEKVTMSCKSSQSLLHSGNQRNYLTWYQQKPGQPPKLLIYWASTRESGVPDRFTGSGSGTDFTLTISSVQAEDLAVYYCQNDYDYPYTFGGGTKLEIKSDPGSGGGGSCPYSNPSLCSGGGGSCPYSNPSLCSGGGGSTTTPAPRPPTPAPTIASQPLSLRPEACRPAAGGAVHTRGLDFACDIYIWAPLAGTCGVLLLSLVITLYCKRGRKKLLYIFKQPFMRPVQTTQEEDGCSCRFPEEEEGGCELRVKFSRSADAPAYQQGQNQLYNELNLGRREEYDVLDKRRGRDPEMGGKPRRKNPQEGLYNELQKDKMAEAYSEIGMKGERRRGKGHDGLYQGLSTATKDTYDALHMQALPPR

SEQ ID NO: 129 - protein, 569 aa, artificial sequence
  25A10v2 CAR with 2 CD20 mimotopes and 1 CD34 epitope
MALPVTALLLPLALLLHAARPGGGGSCPYSNPSLCSGGGGSGGGGSEVQLQQSGAELVRPGASVKLSCTASGFNIKDSLIHWVKQRPEQGLEWIGWIDPEDDKTKYAPKFQDKATLTADTSSNTAYLQLSTLTSEDTAIYYCVSRYINYYFAYWGQGTTLTVSSGGGGSGGGGSGGGGDIVMTQSPSSLTVTAGEKVTMSCKSSQSLLHSGNQRNYLTWYQQKPGQPPKLLIYWASTRESGVPDRFTGSGSGTDFTLTISSVQAEDLAVYYCQNDYDYPYTFGGGTKLEIKGSGGGGSCPYSNPSLCSGGGGSELPTQGTFSNVSTNVSPAKPTTTACPYSNPSLCTTTPAPRPPTPAPTIASQPLSLRPEACRPAAGGAVHTRGLDFACDIYIWAPLAGTCGVLLLSLVITLYCKRGRKKLLYIFKQPFMRPVQTTQEEDGCSCRFPEEEEGGCELRVKFSRSADAPAYQQGQNQLYNELNLGRREEYDVLDKRRGRDPEMGGKPRRKNPQEGLYNELQKDKMAEAYSEIGMKGERRRGKGHDGLYQGLSTATKDTYDALHMQALPPR

SEQ ID NO: 130 - protein, 501 aa, artificial sequence
  25A10v1 CAR with 2 CD20 mimotopes
MALPVTALLLPLALLLHAARPEVQLQQSGAELVRPGASVKLSCTASGFNIKDSLIHWVKQRPEQGLEWIGWIDPEDDKTKYAPKFQDKATLTADTSSNTAYLQLSTLTSEDTAIYYCVSRYINYYFAYWGQGTTLTVSSGGGGSGGGGSGGGGSDIVMTQSPSSLTVTAGEKVTMSCKSSQSLLHSGNQRNYLTWYQQKPGQPPKLLIYWASTRESGVPDRFTGSGSGTDFTLTISSVQAEDLAVYYCQNDYDYPYTFGGGTKLEIKSDPGSGGGGSCPYSNPSLCSGGGGSCPYSNPSLCSGGGGSGLAVSTISSFFPPGYQIYIWAPLAGTCGVLLLSLVITLYCKRGRKKLLYIFKQPFMRPVQTTQEEDGCSCRFPEEEEGGCELRVKFSRSADAPAYQQGQNQLYNELNLGRREEYDVLDKRRGRDPEMGGKPRRKNPQEGLYNELQKDKMAEAYSEIGMKGERRRGKGHDGLYQGLSTATKDTYDALHMQALPPR

SEQ ID NO: 131 - protein, 541 aa, artificial sequence
  25A10v1 CAR with 2 CD20 mimotopes and 1 CD34 epitope
MALPVTALLLPLALLLHAARPGGGGSCPYSNPSLCSGGGGSGGGGSEVQLQQSGAELVRPGASVKLSCTASGFNIKDSLIHWVKQRPEQGLEWIGWIDPEDDKTKYAPKFQDKATLTADTSSNTAYLQLSTLTSEDTAIYYCVSRYINYYFAYWGQGTTLTVSSGGGGSGGGGSGGGGSDIVMTQSPSSLTVTAGEKVTMSCKSSQSLLHSGNQRNYLTWYQQKPGQPPKLLIYWASTRESGVPDRFTGSGSGTDFTLTISSVQAEDLAVYYCQNDYDYPYTFGGGTKLEIKGSGGGGSCPYSNPSLCSGGGGSELPTQGTFSNVSTNVSPAKPTTTACPYSNPSLCGLAVSTISSFFPPGYQIYIWAPLAGTCGVLLLSLVITLYCKRGRKKLLYIFKQPFMRPVQTTQEEDGCSCRFPEEEEGGCELRVKFSRSADAPAYQQGQNQLYNELNLGRREEYDVLDKRRGRDPEMGGKPRRKNPQEGLYNELQKDKMAEAYSEIGMKGERRRGKGHDGLYQGLSTATKDTYDALHMQALPPR

SEQ ID NO: 132 - protein, 117 aa, artificial sequence
  VH chain of m2C2
EVKLVESGGGLVQPGGSLKLSCATSGFTFSDYYMFWVRQTPEKRLEWVAYISNGDGNTYYPDTLKGRFTISRDNANNTLYLQMSRLKSEDTAMYYCARSISRYFDVWGAGTTVTVSS

SEQ ID NO: 133 - protein, 107 aa, artificial sequence
  VL chain of m2C2
DIVMTQSPATLSVTPGDRVSLSCRASQSISDFLHWYQQKSHESPRLLIKYVSQSISGIPSRFSGSGSGSDFTLSINSVEPEDVGVYYCQNAHSFPSTFGGGTKLEIK

SEQ ID NO: 134 - protein, 117 aa, artificial sequence
  VH chain of m5G9
EIHLQQSGPELVKPGASVKISCKASGYSFTDYNIYWVKQSHGESLEWVGYIDPYNGGAYYNQKFKAMATLTVDKSSSTAFMHLNSLTSEDSAVYYCARKGVYGLAYWGQGTLVTVSS

SEQ ID NO: 135 - protein, 107 aa, artificial sequence
  VL chain of m5G9
DIQMTQSPASLSVSVGETVTITCRASESIYSNLAWYQQKQGKSPQLLVYASTHLADGVPSRFSGSGSGAQYSLKINSLQSEDFGSYYCQHFWGTPYTFGGGTKLEIK

SEQ ID NO: 136 - protein, 454 aa, artificial sequence
  5G9-V1 CAR
MALPVTALLLPLALLLHAARPEIHLQQSGPELVKPGASVKISCKASGYSFTDYNIYWVKQSHGESLEWVGYIDPYNGGAYYNQKFKAMATLTVDKSSSTAFMHLNSLTSEDSAVYYCARKGVYGLAYWGQGTLVTVSSGGGGSGGGGSGGGGSDIQMTQSPASLSVSVGETVTITCRASESIYSNLAWYQQKQGKSPQLLVYASTHLADGVPSRFSGSGSGAQYSLKINSLQSEDFGSYYCQHFWGTPYTFGGGTKLEIKGLAVSTISSFFPPGYQIYIWAPLAGTCGVLLLSLVITLYCKRGRKKLLYIFKQPFMRPVQTTQEEDGCSCRFPEEEEGGCELRVKFSRSADAPAYQQGQNQLYNELNLGRREEYDVLDKRRGRDPEMGGKPRRKNPQEGLYNELQKDKMAEAYSEIGMKGERRRGKGHDGLYQGLSTATKDTYDALHMQALPPR

SEQ ID NO: 137 - protein, 483 aa, artificial sequence
  5G9-V2 CAR
MALPVTALLLPLALLLHAARPEIHLQQSGPELVKPGASVKISCKASGYSFTDYNIYWVKQSHGESLEWVGYIDPYNGGAYYNQKFKAMATLTVDKSSSTAFMHLNSLTSEDSAVYYCARKGVYGLAYWGQGTLVTVSSGGGGSGGGGSGGGGSDIQMTQSPASLSVSVGETVTITCRASESIYSNLAWYQQKQGKSPQLLVYASTHLADGVPSRFSGSGSGAQYSLKINSLQSEDFGSYYCQHFWGTPYTFGGGTKLEIKTTTPAPRPPTPAPTIASQPLSLRPEACRPAAGGAVHTRGLDFACDIYIWAPLAGTCGVLLLSLVITLYCKRGRKKLLYIFKQPFMRPVQTTQEEDGCSCRFPEEEEGGCELRVKFSRSADAPAYQQGQNQLYNELNLGRREEYDVLDKRRGRDPEMGGKPRRKNPQEGLYNELQKDKMAEAYSEIGMKGERRRGKGHDGLYQGLSTATKDTYDALHMQALPPR

SEQ ID NO: 138 - protein, 669 aa, artificial sequence
  5G9-V3 CAR
MALPVTALLLPLALLLHAARPEIHLQQSGPELVKPGASVKISCKASGYSFTDYNIYWVKQSHGESLEWVGYIDPYNGGAYYNQKFKAMATLTVDKSSSTAFMHLNSLTSEDSAVYYCARKGVYGLAYWGQGTLVTVSSGGGGSGGGGSGGGGSDIQMTQSPASLSVSVGETVTITCRASESIYSNLAWYQQKQGKSPQLLVYASTHLADGVPSRFSGSGSGAQYSLKINSLQSEDFGSYYCQHFWGTPYTFGGGTKLEIKEPKSPDKTHTCPPCPAPPVAGPSVFLFPPKPKDTLMIARTPEVTCVVVDVSHEDPEVKFNWYVDGVEVHNAKTKPREEQYNSTYRVVSVLTVLHQDWLNGKEYKCKVSNKALPAPIEKTISKAKGQPREPQVYTLPPSRDELTKNQVSLTCLVKGFYPSDIAVEWESNGQPENNYKTTPPVLDSDGSFFLYSKLTVDKSRWQQGNVFSCSVMHEALHNHYTQKSLSLSPGKIYIWAPLAGTCGVLLLSLVITLYCKRGRKKLLYIFKQPFMRPVQTTQEEDGCSCRFPEEEEGGCELRVKFSRSADAPAYQQGQNQLYNELNLGRREEYDVLDKRRGRDPEMGGKPRRKNPQEGLYNELQKDKMAEAYSEIGMKGERRRGKGHDGLYQGLSTATKDTYDALHMQALPPR

SEQ ID NO: 139 - protein, 454 aa, artificial sequence
  2C2-V1 CAR
MALPVTALLLPLALLLHAARPEVKLVESGGGLVQPGGSLKLSCATSGFTFSDYYMFWVRQTPEKRLEWVAYISNGDGNTYYPDTLKGRFTISRDNANNTLYLQMSRLKSEDTAMYYCARSISRYFDVWGAGTTVTVSSGGGGSGGGGSGGGGSDIVMTQSPATLSVTPGDRVSLSCRASQSISDFLHWYQQKSHESPRLLIKYVSQSISGIPSRFSGSGSGSDFTLSINSVEPEDVGVYYCQNAHSFPSTFGGGTKLEIKGLAVSTISSFFPPGYQIYIWAPLAGTCGVLLLSLVITLYCKRGRKKLLYIFKQPFMRPVQTTQEEDGCSCRFPEEEEGGCELRVKFSRSADAPAYQQGQNQLYNELNLGRREEYDVLDKRRGRDPEMGGKPRRKNPQEGLYNELQKDKMAEAYSEIGMKGERRRGKGHDGLYQGLSTATKDTYDALHMQALPPR

SEQ ID NO: 140 - protein, 483 aa, artificial sequence
  2C2-V2 CAR
MALPVTALLLPLALLLHAARPEVKLVESGGGLVQPGGSLKLSCATSGFTFSDYYMFWVRQTPEKRLEWVAYISNGDGNTYYPDTLKGRFTISRDNANNTLYLQMSRLKSEDTAMYYCARSISRYFDVWGAGTTVTVSSGGGGSGGGGSGGGGSDIVMTQSPATLSVTPGDRVSLSCRASQSISDFLHWYQQKSHESPRLLIKYVSQSISGIPSRFSGSGSGSDFTLSINSVEPEDVGVYYCQNAHSFPSTFGGGTKLEIKTTTPAPRPPTPAPTIASQPLSLRPEACRPAAGGAVHTRGLDFACDIYIWAPLAGTCGVLLLSLVITLYCKRGRKKLLYIFKQPFMRPVQTTQEEDGCSCRFPEEEEGGCELRVKFSRSADAPAYQQGQNQLYNELNLGRREEYDVLDKRRGRDPEMGGKPRRKNPQEGLYNELQKDKMAEAYSEIGMKGERRRGKGHDGLYQGLSTATKDTYDALHMQALPPR

SEQ ID NO: 141 - protein, 669 aa, artificial sequence
  2C2-V3 CAR
MALPVTALLLPLALLLHAARPEVKLVESGGGLVQPGGSLKLSCATSGFTFSDYYMFWVRQTPEKRLEWVAYISNGDGNTYYPDTLKGRFTISRDNANNTLYLQMSRLKSEDTAMYYCARSISRYFDVWGAGTTVTVSSGGGGSGGGGSGGGGSDIVMTQSPATLSVTPGDRVSLSCRASQSISDFLHWYQQKSHESPRLLIKYVSQSISGIPSRFSGSGSGSDFTLSINSVEPEDVGVYYCQNAHSFPSTFGGGTKLEIKEPKSPDKTHTCPPCPAPPVAGPSVFLFPPKPKDTLMIARTPEVTCVVVDVSHEDPEVKFNWYVDGVEVHNAKTKPREEQYNSTYRVVSVLTVLHQDWLNGKEYKCKVSNKALPAPIEKTISKAKGQPREPQVYTLPPSRDELTKNQVSLTCLVKGFYPSDIAVEWESNGQPENNYKTTPPVLDSDGSFFLYSKLTVDKSRWQQGNVFSCSVMHEALHNHYTQKSLSLSPGKIYIWAPLAGTCGVLLLSLVITLYCKRGRKKLLYIFKQPFMRPVQTTQEEDGCSCRFPEEEEGGCELRVKFSRSADAPAYQQGQNQLYNELNLGRREEYDVLDKRRGRDPEMGGKPRRKNPQEGLYNELQKDKMAEAYSEIGMKGERRRGKGHDGLYQGLSTATKDTYDALHMQALPPR

SEQ ID NO: 142 - protein, 118 aa, artificial sequence
  VH chain of m9E2
EVQLQQSGPELEKPGASVKISCKASGYSFTDYNMNWVKQSNGKSLEWIGNIDPDYGGTTYNQKFKGKATLTVDKSSSTAYMQLRSLTSEDSAVYYCARSGYRYGFVYWGQGTLVTVSA

SEQ ID NO: 143 - protein, 112 aa, artificial sequence
  VL chain of m9E2
DIVMTQAAFSNPVTLGTSASISCRSSKSLLHSNGITYLYWYLQKPGQSPQLLIYQMSNLASGVPDRFSSSGSGTDFTLRISRVEAEDVGVYYCAQNLELPWTFGGGTKLEIK

SEQ ID NO: 144 - protein, 115 aa, artificial sequence
  VH chain of m28B9
EVQLQQSGAELVRPGASVKLSCTASGFNIKDDYLHWMKQRPEQGLEWIGRIDPANGNTKSDPKFQDKATIDADTSSNTAYLQLNSLTSEDTAVYYCAKGPWFPYWGQGTLVTVSA

SEQ ID NO: 145 - protein, 107 aa, artificial sequence
  VL chain of m28B9
DIQMTQSPASQSASLGESVTITCLASQTIGTWLAWYQQKPGKSPQLLIYAATSLADGVPSRFSGSGSGTKFSFKISSLQAEDFVSYHCQQLYRTPLTFGGGTKLEIK

SEQ ID NO: 146 - protein, 120 aa, artificial sequence
  VH chain of m26D8
QVQLQQPGAEMVRPGASVKLSCKASGYTFTDYWMHWVKQRPGQGLEWIGKIDPSDSETHYHQKFKDKATLTVDKSSSTAYLQFKSLTSEDSAVHYCAREGIWLRYAMDYWGQGTSVTVSS

SEQ ID NO: 147 - protein, 107 aa, artificial sequence
  VL chain of m26D8
DIVMTQSQKFMSTSVGDRVSVTCKASQNVGTNVAWYQQKPGQSPKALIYSASYRYSGVPDRFTGSGSGTDFTLTVSSVQSEDLAEYFCQQYNSYPYTFGGGTKLEIK

SEQ ID NO: 148 - protein, 121 aa, artificial sequence
  VH chain of m15D1
EVQLQQSGPELVKPGASVKMSCRASGYSITDYNMHWVKQSHGKSLEWIGYIDPDNGATNNNQKFKGKATLTVDKSSSTAYMQLSSLTSEDSAVYYCARSEGYQYYYAMDYWGQGTSVTVSS

SEQ ID NO: 149 - protein, 112 aa, artificial sequence
  VL chain of m15D1
DIVMTQAAFSNPVALGTSASISCSSSKSLLHSNGITYLHWYLQRPGQSPQLLIYRMSNLASGVPDRFSGSGSGTDFTLRISRVEAEDVGVYYCAQMVERPWTFGGGTKLEIK

SEQ ID NO: 150 - protein, 120 aa, artificial sequence
  VH chain of m23F2
QVQVQQPGAELVKPGASVKLSCKASGYTFTSYWINWVKQRPGQGLEWIGNIYPGSSSTNHNEKFKSKATLTVDTSSSTAYMQLSSLTSDDSAVYYCARRGSSPSYTMDYWGQGTSVTVSS

SEQ ID NO: 151 - protein, 111 aa, artificial sequence
  VL chain of m23F2
DIVLTQSPASLAVALGQRATISCRASKSVSTFGYSYMHWYQQKPGQAPKLLIYLASNLESGVPARFSGSGSGTDFTLKIHPVEEEDAATYYCLHSRELPWTFGGGTKLEIK